European Patent Application EP 4 497 759 A1, published January 29, 2025. Title: CHIMERIC ANTIGEN RECEPTOR TARGETING GPRC5D AND APPLICATION THEREOF. Applicant: Oricell Therapeutics Co.,Ltd. The sequence listing filed with the application follows.

SEQUENCE LISTING (40 sequences)

SEQ ID NO: 1 - protein, 21 aa, synthetic construct
  REGION 1..21: note = CD8 signal peptide
MALPVTALLLPLALLLHAARP

SEQ ID NO: 2 - protein, 45 aa, synthetic construct
  REGION 1..45: note = CD8 hinge region
TTTPAPRPPTPAPTIASQPLSLRPEACRPAAGGAVHTRGLDFACD

SEQ ID NO: 3 - protein, 24 aa, synthetic construct
  REGION 1..24: note = CD8 transmembrane region
IYIWAPLAGTCGVLLLSLVITLYC

SEQ ID NO: 4 - protein, 42 aa, synthetic construct
  REGION 1..42: note = CD137(4-1BB) co-stimulatory region
KRGRKKLLYIFKQPFMRPVQTTQEEDGCSCRFPEEEEGGCEL

SEQ ID NO: 5 - protein, 112 aa, synthetic construct
  REGION 1..112: note = CD3zeta intracellular signaling domain
RVKFSRSADAPAYQQGQNQLYNELNLGRREEYDVLDKRRGRDPEMGGKPRRKNPQEGLYNELQKDKMAEAYSEIGMKGERRRGKGHDGLYQGLSTATKDTYDALHMQALPPR

SEQ ID NO: 6 - protein, 18 aa, synthetic construct
  REGION 1..18: note = T2A
EGRGSLLTCGDVEENPGP

SEQ ID NO: 7 - protein, 398 aa, synthetic construct
  REGION 1..398: note = ori
MGAVLRSLLACSFCVLLRAEQKLISEEDLEPPTCSPQQFTCFTGEIDCIPVAWRCDGFTECEDHSDELNCPVCSESQFQCASGQCIDGALRCNGDANCQDKSDEKNCEVLCLIDQFRCANGQCIGKHKKCDHNVDCSDKSDELDCYPTEEPAPQATNTVGSVIGVIVTIFVSGTVYFICQRMLCPRMKGDGETMTNDYVVHGPASVPLGYVPHPSSLSGSLPGMSRGKSMISSLSIMGGSSGPPYDRAHVTGASSSSSSSTKGTYFPAILNPPPSPATERSHYTMEFGYSSNSPSTHRSYSYRPYSYRHFAPPTTPCSTDVCDSDYAPSRRMTSVATAKGYTSDLNYDSEPVPPPPTPRSQYLSAEENYESCPPSPYTERSYSHHLYPPPPSPCTDSS

SEQ ID NO: 8 - protein, 8 aa, synthetic construct
  REGION 1..8: note = 3B5 HCDR1
GFIFSRYG

SEQ ID NO: 9 - protein, 8 aa, synthetic construct
  REGION 1..8: note = 3B5 HCDR2
INWSDGTT

SEQ ID NO: 10 - protein, 14 aa, synthetic construct
  REGION 1..14: note = 3B5HCDR3
AADRRLRSQTGYDY

SEQ ID NO: 11 - protein, 25 aa, synthetic construct [sequence omitted]

SEQ ID NO: 12 - protein, 17 aa, synthetic construct
  REGION 1..17: note = 3B5, 3E7 H-FR2
MGWFRQAPGKGRELVAA

SEQ ID NO: 13 - protein, 38 aa, synthetic construct
  REGION 1..38: note = 3B5, 3E7, 4A2 H-FR3
YYPDSVEGRFTISRDNAKRMVYLQMNSLRAEDTAVYYC

SEQ ID NO: 14 - protein, 11 aa, synthetic construct
  REGION 1..11: note = 3B5, 3E7, 4A2, 4B3 H-FR4
WGQGTQVTVSS

SEQ ID NO: 15 - protein, 121 aa, synthetic construct
  REGION 1..121: note = 3B5 VHH
EVQLVESGGGLVQPGGSLRLSCAASGFIFSRYGMGWFRQAPGKGRELVAAINWSDGTTYYPDSVEGRFTISRDNAKRMVYLQMNSLRAEDTAVYYCAADRRLRSQTGYDYWGQGTQVTVSS

SEQ ID NO: 16 - protein, 8 aa, synthetic construct
  REGION 1..8: note = 3E7 HCDR1
GRIFSRDA

SEQ ID NO: 17 - protein, 8 aa, synthetic construct
  REGION 1..8: note = 3E7 HCDR2
INSSGGNT

SEQ ID NO: 18 - protein, 17 aa, synthetic construct
  REGION 1..17: note = 3E7 HCDR3
AARGVRWTSTTAYGYNY

SEQ ID NO: 19 - protein, 124 aa, synthetic construct
  REGION 1..124: note = 3E7 VHH
EVQLVESGGGLVQPGGSLRLSCAASGRIFSRDAMGWFRQAPGKGRELVAAINSSGGNTYYPDSVEGRFTISRDNAKRMVYLQMNSLRAEDTAVYYCAARGVRWTSTTAYGYNYWGQGTQVTVSS

SEQ ID NO: 20 - protein, 8 aa, synthetic construct
  REGION 1..8: note = 4A2 HCDR1
GFIFSRYD

SEQ ID NO: 21 - protein, 8 aa, synthetic construct
  REGION 1..8: note = 4A2 HCDR2
ITWGGGST

SEQ ID NO: 22 - protein, 17 aa, synthetic construct
  REGION 1..17: note = 4A2 HCDR3
AARSASAYRTGRLEYNY

SEQ ID NO: 23 - protein, 17 aa, synthetic construct
  REGION 1..17: note = 4A2 H-FR2
MGWFRQAPGKGRELVAV

SEQ ID NO: 24 - protein, 124 aa, synthetic construct
  REGION 1..124: note = 4A2 VHH
EVQLVESGGGLVQPGGSLRLSCAASGFIFSRYDMGWFRQAPGKGRELVAVITWGGGSTYYPDSVEGRFTISRDNAKRMVYLQMNSLRAEDTAVYYCAARSASAYRTGRLEYNYWGQGTQVTVSS

SEQ ID NO: 25 - protein, 8 aa, synthetic construct
  REGION 1..8: note = 4B3 HCDR1
GLIFSRYV

SEQ ID NO: 26 - protein, 8 aa, synthetic construct
  REGION 1..8: note = 4B3 HCDR2
INSSGGST

SEQ ID NO: 27 - protein, 14 aa, synthetic construct
  REGION 1..14: note = 4B3 HCDR3
AASSRTSTTRGYNY

SEQ ID NO: 28 - protein, 17 aa, synthetic construct
  REGION 1..17: note = 4B3 H-FR2
MGWFRQAPGKGRELVAF

SEQ ID NO: 29 - protein, 38 aa, synthetic construct
  REGION 1..38: note = 4B3 H-FR3
NYPDSVEGRFTISRDNAKRMVYLQMNSLRAEDTAVYYC

SEQ ID NO: 30 - protein, 121 aa, synthetic construct
  REGION 1..121: note = 4B3 VHH
EVQLVESGGGLVQPGGSLRLSCAASGLIFSRYVMGWFRQAPGKGRELVAFINSSGGSTNYPDSVEGRFTISRDNAKRMVYLQMNSLRAEDTAVYYCAASSRTSTTRGYNYWGQGTQVTVSS

SEQ ID NO: 31 - protein, 927 aa, synthetic construct
  REGION 1..927: note = OriCAR-DG501M
MALPVTALLLPLALLLHAARPEVQLVESGGGLVQPGGSLRLSCAASGFIFSRYGMGWFRQAPGKGRELVAAINWSDGTTYYPDSVEGRFTISRDNAKRMVYLQMNSLRAEDTAVYYCAADRRLRSQTGYDYWGQGTQVTVSSGGGGSGGGGSGGGGSGGGGSGGGGSEVQLVESGGGLVQPGGSLRLSCAASGFIFSRYGMGWFRQAPGKGRELVAAINWSDGTTYYPDSVEGRFTISRDNAKRMVYLQMNSLRAEDTAVYYCAADRRLRSQTGYDYWGQGTQVTVSSTTTPAPRPPTPAPTIASQPLSLRPEACRPAAGGAVHTRGLDFACDIYIWAPLAGTCGVLLLSLVITLYCKRGRKKLLYIFKQPFMRPVQTTQEEDGCSCRFPEEEEGGCELRVKFSRSADAPAYQQGQNQLYNELNLGRREEYDVLDKRRGRDPEMGGKPRRKNPQEGLYNELQKDKMAEAYSEIGMKGERRRGKGHDGLYQGLSTATKDTYDALHMQALPPREGRGSLLTCGDVEENPGPMGAVLRSLLACSFCVLLRAEQKLISEEDLEPPTCSPQQFTCFTGEIDCIPVAWRCDGFTECEDHSDELNCPVCSESQFQCASGQCIDGALRCNGDANCQDKSDEKNCEVLCLIDQFRCANGQCIGKHKKCDHNVDCSDKSDELDCYPTEEPAPQATNTVGSVIGVIVTIFVSGTVYFICQRMLCPRMKGDGETMTNDYVVHGPASVPLGYVPHPSSLSGSLPGMSRGKSMISSLSIMGGSSGPPYDRAHVTGASSSSSSSTKGTYFPAILNPPPSPATERSHYTMEFGYSSNSPSTHRSYSYRPYSYRHFAPPTTPCSTDVCDSDYAPSRRMTSVATAKGYTSDLNYDSEPVPPPPTPRSQYLSAEENYESCPPSPYTERSYSHHLYPPPPSPCTDSS

SEQ ID NO: 32 - protein, 917 aa, synthetic construct
  REGION 1..917: note = OriCAR-DG517M
MALPVTALLLPLALLLHAARPEVQLVESGGGLVQPGGSLRLSCAASGFIFSRYGMGWFRQAPGKGRELVAAINWSDGTTYYPDSVEGRFTISRDNAKRMVYLQMNSLRAEDTAVYYCAADRRLRSQTGYDYWGQGTQVTVSSEAAAKEAAAKEAAAKEVQLVESGGGLVQPGGSLRLSCAASGFIFSRYGMGWFRQAPGKGRELVAAINWSDGTTYYPDSVEGRFTISRDNAKRMVYLQMNSLRAEDTAVYYCAADRRLRSQTGYDYWGQGTQVTVSSTTTPAPRPPTPAPTIASQPLSLRPEACRPAAGGAVHTRGLDFACDIYIWAPLAGTCGVLLLSLVITLYCKRGRKKLLYIFKQPFMRPVQTTQEEDGCSCRFPEEEEGGCELRVKFSRSADAPAYQQGQNQLYNELNLGRREEYDVLDKRRGRDPEMGGKPRRKNPQEGLYNELQKDKMAEAYSEIGMKGERRRGKGHDGLYQGLSTATKDTYDALHMQALPPREGRGSLLTCGDVEENPGPMGAVLRSLLACSFCVLLRAEQKLISEEDLEPPTCSPQQFTCFTGEIDCIPVAWRCDGFTECEDHSDELNCPVCSESQFQCASGQCIDGALRCNGDANCQDKSDEKNCEVLCLIDQFRCANGQCIGKHKKCDHNVDCSDKSDELDCYPTEEPAPQATNTVGSVIGVIVTIFVSGTVYFICQRMLCPRMKGDGETMTNDYVVHGPASVPLGYVPHPSSLSGSLPGMSRGKSMISSLSIMGGSSGPPYDRAHVTGASSSSSSSTKGTYFPAILNPPPSPATERSHYTMEFGYSSNSPSTHRSYSYRPYSYRHFAPPTTPCSTDVCDSDYAPSRRMTSVATAKGYTSDLNYDSEPVPPPPTPRSQYLSAEENYESCPPSPYTERSYSHHLYPPPPSPCTDSS

SEQ ID NO: 33 - protein, 17 aa, synthetic construct
  REGION 1..17: note = 3B5 HCDR3; 3E7 HCDR3; 4A2 HCDR3; 4B3 HCDR3
  SITE 3: note = misc_feature - Xaa = Arg, Ser or does not exist
  SITE 4: note = misc_feature - Xaa = Asp, Gly or Ser
  SITE 5: note = misc_feature - Xaa = Ala, Arg, Val or does not exist
  SITE 6: note = misc_feature - Xaa = Arg or Ser
  SITE 7: note = misc_feature - Xaa = Ala, Leu, Trp or does not exist
  SITE 8: note = misc_feature - Xaa = Arg, Thr or Tyr
  SITE 9: note = misc_feature - Xaa = Arg or Ser
  SITE 10: note = misc_feature - Xaa = Gln or Thr
  SITE 11: note = misc_feature - Xaa = Gly or Thr
  SITE 12: note = misc_feature - Xaa = Ala, Arg or does not exist
  SITE 13: note = misc_feature - Xaa = Leu, Tyr or does not exist
  SITE 14: note = misc_feature - Xaa = Glu or Gly
  SITE 16: note = misc_feature - Xaa = Asp or Asn
AAXXXXXXXXXXXXYXY

SEQ ID NO: 34 - skipped

SEQ ID NO: 35 - protein, 8 aa, synthetic construct
  REGION 1..8: note = 3B5 HCDR1; 3E7 HCDR1; 4A2 HCDR1; 4B3 HCDR1
  SITE 2: note = misc_feature - Xaa = Phe, Leu or Arg
  SITE 7: note = misc_feature - Xaa = Asp or Tyr
  SITE 8: note = misc_feature - Xaa = Ala, Asp, Gly or Val
GXIFSRXX

SEQ ID NO: 36 - protein, 300 aa, Macaca fascicularis
MYKDCIESTGDYFLPCDSEGPWGIVLESLAILGIVVTILLLLAFLFLMRKIQDCSQWNVLPTQLLFLLSVLGLFGLAFAFIIQLNQQTAPVRYFLFGVLFALCFSCLLAHASNLVKLVRGRVSFSWTTILCIAIGCSLLQVIIAIEYVTLIMTRGMMFVHMTPYQLNVDFVVLLVYVLFLMALTFFVSKATFCGPCENWKQHGRLIFITVLFSIIIWVVWISMLLRGNPQFQRQPQWDDPVVCIALVTNAWVFLLLYIVPELCILYRSCRQECPSQGHACPVTAYQRSFQVENQELSRDC

SEQ ID NO: 37 - protein, 344 aa, Mus musculus
MYEDCVKSTEDYYLFCDNEGPWAIVLESLAVIGIVVTILLLLAFLFLMRKVQDCSQWNVLPTQFLFLLAVLGLFGLTFAFIIQLNHQTAPVRYFLFGVLFAICFSCLLAHASNLVKLVRGRVSFCWTTILFIAIGVSLLQTIIAIEYVTLIMTRGLMFEHMTPYQLNVDFVCLLIYVLFLMALTFFVSKATFCGPCENWKQHGRLIFATVLVSIIIWVVWISMLLRGNPQLQRQPHWDDAVICIGLVTNAWVFLLIYIIPELSILYRSCRQECPTQGNVCQVPVYQRSFRMDTQEPTRARDSDGAQEDVALTAYGTPIQLQSADPSREYLIPSATLSPQQDAGL

SEQ ID NO: 38 - protein, 357 aa, Homo sapiens
MATTVPDGCRNGLKSKYYRLCDKAEAWGIVLETVATAGVVTSVAFMLTLPILVCKVQDSNRRKMLPTQFLFLLGVLGIFGLTFAFIIGLDGSTGPTRFFLFGILFSICFSCLLAHAVSLTKLVRGRKPLSLLVILGLAVGFSLVQDVIAIEYIVLTMNRTNVNVFSELSAPRRNEDFVLLLTYVLFLMALTFLMSSFTFCGSFTGWKRHGAHIYLTMLLSIAIWVAWITLLMLPDFDRRWDDTILSSALAANGWVFLLAYVSPEFWLLTKQRNPMDYPVEDAFCKPQLVKKSYGVENRAYSQEEITQGFEETGDTLYAPYSTHFQLQNQPPQKEFSIPRAHAWPSPYKDYEVKKEGS

SEQ ID NO: 39 - protein, 5 aa, synthetic construct
  REGION 1..5: note = G4S linker (repeat unit)
GGGGS

SEQ ID NO: 40 - protein, 5 aa, synthetic construct
  REGION 1..5: note = EAAAK linker (repeat unit)
EAAAK